European Patent Application EP 4 674 438 A1, published January 7, 2026. Title: Ａｎ antibody-drug conjugate comprising anti-CD138 antibody. Applicant: Taiho Pharmaceutical Co., Ltd. The sequence listing filed with the application follows.

SEQUENCE LISTING (50 sequences)

SEQ ID NO: 1 - protein, 5 aa, synthetic construct
  REGION 1..5: note = Amino acid sequence of CDR1 of heavy chain from antibody 1 to antibody 12
NYWIE

SEQ ID NO: 2 - protein, 17 aa, synthetic construct
  REGION 1..17: note = Amino acid sequence of CDR2 of heavy chain from antibody 1 to antibody 12
EILPGTGRTIYNEKFKG

SEQ ID NO: 3 - protein, 13 aa, synthetic construct
  REGION 1..13: note = Amino acid sequence of CDR3 of heavy chain from antibody 1 to antibody 12
RDYYGNFYYAMDY

SEQ ID NO: 4 - protein, 11 aa, synthetic construct
  REGION 1..11: note = Amino acid sequence of CDR1 of light chain from antibody 1 to antibody 12
SASQGINNYLN

SEQ ID NO: 5 - protein, 7 aa, synthetic construct
  REGION 1..7: note = Amino acid sequence of CDR2 of light chain from antibody 1 to antibody 12
YTSTLQS

SEQ ID NO: 6 - protein, 9 aa, synthetic construct
  REGION 1..9: note = Amino acid sequence of CDR3 of light chain from antibody 1 to antibody 12
QQYSKLPRT

SEQ ID NO: 7 - DNA, 366 bp, synthetic construct
  misc_feature 1..366: note = Nucleotide sequence of cDNA encoding the variable region of the heavy chain of antibody 1
  source 1..366: mol_type = other DNA
caggttcagctgcagcagtctggcagcgagcttatgatgcctggcgcctccgtgaagatcagctgtaaagccaccggctacaccttcagcaactactggatcgagtgggtcaagcagaggcctggccatggactggaatggatcggagagatcctgcctggcaccggcagaaccatctacaacgagaagttcaagggcaaagccaccttcaccgccgacatcagcagcaacacagtgcagatgcagctgagcagcctgaccagcgaagatagcgccgtgtactactgcgccagacgggactactacggcaacttctactacgccatggattactggggccagggcaccctggttacagtgtctagc

SEQ ID NO: 8 - protein, 122 aa, synthetic construct
  REGION 1..122: note = Amino acid sequence of the variable region of the heavy chain of antibody 1
QVQLQQSGSELMMPGASVKISCKATGYTFSNYWIEWVKQRPGHGLEWIGEILPGTGRTIYNEKFKGKATFTADISSNTVQMQLSSLTSEDSAVYYCARRDYYGNFYYAMDYWGQGTLVTVSS

SEQ ID NO: 9 - DNA, 321 bp, synthetic construct
  misc_feature 1..321: note = Nucleotide sequence of cDNA encoding the variable region of the light chain of antibody 1 and antibody 2
  source 1..321: mol_type = other DNA
gacatccagatgacccagagcaccagcagcctgtctgcctctctgggcgatagagtgaccatcagctgtagcgccagccagggcatcaacaactacctgaactggtatcagcagaaacccgacggcaccgtggaactgctgatctactacaccagcacactgcagagcggcgtgcccagcagattttctggctctggcagcggcaccgactacagcctgacaatcagcaacctggaacctgaggacatcggcacctactactgccagcagtacagcaagctgcccagaacctttggcggaggcaccaagctggaaatcaag

SEQ ID NO: 10 - protein, 107 aa, synthetic construct
  REGION 1..107: note = Amino acid sequence of the variable region of the light chain of antibody 1 and antibody 2
DIQMTQSTSSLSASLGDRVTISCSASQGINNYLNWYQQKPDGTVELLIYYTSTLQSGVPSRFSGSGSGTDYSLTISNLEPEDIGTYYCQQYSKLPRTFGGGTKLEIK

SEQ ID NO: 11 - DNA, 366 bp, synthetic construct
  misc_feature 1..366: note = Nucleotide sequence of cDNA encoding the variable region of the heavy chain of antibody 2
  source 1..366: mol_type = other DNA
caggttcagctgcagcagtctggcagcgagcttatgatgcctggcgcctccgtgaagatcagctgtaaagccaccggctacaccttcagcaactactggatcgagtgggtcaagcagaggcctggccatggactggaatggatcggagagatcctgcctggcaccggcagaaccatctacaacgagaagttcaagggcaaagccaccttcaccgccgacatcagcagcaacacagtgcagatgcagctgagcagcctgaccagcgaagatagcgccgtgtactactgcgccagacgggactactacggcaacttctactacgccatggattactggggccagggcaccagcgtgacagtgtctagc

SEQ ID NO: 12 - protein, 122 aa, synthetic construct
  REGION 1..122: note = Amino acid sequence of the variable region of the heavy chain of antibody 2
QVQLQQSGSELMMPGASVKISCKATGYTFSNYWIEWVKQRPGHGLEWIGEILPGTGRTIYNEKFKGKATFTADISSNTVQMQLSSLTSEDSAVYYCARRDYYGNFYYAMDYWGQGTSVTVSS

SEQ ID NO: 13 - DNA, 366 bp, synthetic construct
  misc_feature 1..366: note = Nucleotide sequence of cDNA encoding the variable region of the heavy chain of antibody 3 and antibody 10
  source 1..366: mol_type = other DNA
caggtccagctcgtccagtccggcgccgaggtcaagaagcccggctcctccgtcaaggtctcctgcaaggcctccggctacaccttctccaactactggatcgagtgggtccgccaggcccccggccagggcctcgagtggatcggcgagatcctccccggcaccggccgcaccatctacaacgagaagttcaagggccgcgccaccttcaccgccgacatctccacctccaccgcctacatggagctctcctccctccgctccgaggacaccgccgtctactactgcgcccgccgcgactactacggcaacttctactacgccatggactactggggccagggcaccctcgtcaccgtctcctcc

SEQ ID NO: 14 - protein, 122 aa, synthetic construct
  REGION 1..122: note = Amino acid sequence of the variable region of the heavy chain of antibody 3 and antibody 10
QVQLVQSGAEVKKPGSSVKVSCKASGYTFSNYWIEWVRQAPGQGLEWIGEILPGTGRTIYNEKFKGRATFTADISTSTAYMELSSLRSEDTAVYYCARRDYYGNFYYAMDYWGQGTLVTVSS

SEQ ID NO: 15 - DNA, 321 bp, synthetic construct
  misc_feature 1..321: note = Nucleotide sequence of cDNA encoding the variable region of the light chain of antibody 3, 4, 5, 6, 10, 11, and 12
  source 1..321: mol_type = other DNA
gacatccagatgacccagtccccctcctccctctccgcctccgtcggcgaccgcgtcaccatcacctgctccgcctcccagggcatcaacaactacctcaactggtaccagcagaagcccggcaaggcccccaagctcctcatctactacacctccaccctccagtccggcgtcccctcccgcttctccggctccggctccggcaccgactacaccctcaccatctcctccctccagcccgaggacttcgccacctactactgccagcagtactccaagctcccccgcaccttcggcggcggcaccaaggtcgagatcaag

SEQ ID NO: 16 - protein, 107 aa, synthetic construct
  REGION 1..107: note = Amino acid sequence of the variable region of the light chain of antibody 3, 4, 5, 6, 10, 11, and 12
DIQMTQSPSSLSASVGDRVTITCSASQGINNYLNWYQQKPGKAPKLLIYYTSTLQSGVPSRFSGSGSGTDYTLTISSLQPEDFATYYCQQYSKLPRTFGGGTKVEIK

SEQ ID NO: 17 - DNA, 366 bp, synthetic construct
  misc_feature 1..366: note = Nucleotide sequence of cDNA encoding the variable region of the heavy chain of antibody 4, 7, and 11
  source 1..366: mol_type = other DNA
caggtccagctcgtccagtccggcgccgaggtcaagaagcccggctcctccgtcaaggtctcctgcaaggcctccggctacaccttctccaactactggatcgagtgggtccgccaggcccccggccagggcctcgagtggatcggcgagatcctccccggcaccggccgcaccatctacaacgagaagttcaagggccgcgtcaccttcaccgccgacatctccacctccaccgcctacatggagctctcctccctccgctccgaggacaccgccgtctactactgcgcccgccgcgactactacggcaacttctactacgccatggactactggggccagggcaccctcgtcaccgtctcctcc

SEQ ID NO: 18 - protein, 122 aa, synthetic construct
  REGION 1..122: note = Amino acid sequence of the variable region of the heavy chain of antibody 4, 7, and 11
QVQLVQSGAEVKKPGSSVKVSCKASGYTFSNYWIEWVRQAPGQGLEWIGEILPGTGRTIYNEKFKGRVTFTADISTSTAYMELSSLRSEDTAVYYCARRDYYGNFYYAMDYWGQGTLVTVSS

SEQ ID NO: 19 - DNA, 366 bp, synthetic construct
  misc_feature 1..366: note = Nucleotide sequence of cDNA encoding the variable region of the heavy chain of antibody 5 and antibody 8
  source 1..366: mol_type = other DNA
caggtccagctcgtccagtccggcgccgaggtcaagaagcccggctcctccgtcaaggtctcctgcaaggcctccggctacaccttctccaactactggatcgagtgggtccgccaggcccccggccagggcctcgagtggatcggcgagatcctccccggcaccggccgcaccatctacaacgagaagttcaagggccgcgccaccttcaccgccgacgagtccacctccaccgcctacatggagctctcctccctccgctccgaggacaccgccgtctactactgcgcccgccgcgactactacggcaacttctactacgccatggactactggggccagggcaccctcgtcaccgtctcctcc

SEQ ID NO: 20 - protein, 122 aa, synthetic construct
  REGION 1..122: note = Amino acid sequence of the variable region of the heavy chain of antibody 5 and antibody 8
QVQLVQSGAEVKKPGSSVKVSCKASGYTFSNYWIEWVRQAPGQGLEWIGEILPGTGRTIYNEKFKGRATFTADESTSTAYMELSSLRSEDTAVYYCARRDYYGNFYYAMDYWGQGTLVTVSS

SEQ ID NO: 21 - DNA, 366 bp, synthetic construct
  misc_feature 1..366: note = Nucleotide sequence of cDNA encoding the variable region of the heavy chain of antibody 6, 9, and 12
  source 1..366: mol_type = other DNA
caggtccagctcgtccagtccggcgccgaggtcaagaagcccggctcctccgtcaaggtctcctgcaaggcctccggctacaccttctccaactactggatcgagtgggtccgccaggcccccggccagggcctcgagtggatcggcgagatcctccccggcaccggccgcaccatctacaacgagaagttcaagggccgcgtcaccttcaccgccgacgagtccacctccaccgcctacatggagctctcctccctccgctccgaggacaccgccgtctactactgcgcccgccgcgactactacggcaacttctactacgccatggactactggggccagggcaccctcgtcaccgtctcctcc

SEQ ID NO: 22 - protein, 122 aa, synthetic construct
  REGION 1..122: note = Amino acid sequence of the variable region of the heavy chain of antibody 6, 9, and 12
QVQLVQSGAEVKKPGSSVKVSCKASGYTFSNYWIEWVRQAPGQGLEWIGEILPGTGRTIYNEKFKGRVTFTADESTSTAYMELSSLRSEDTAVYYCARRDYYGNFYYAMDYWGQGTLVTVSS

SEQ ID NO: 23 - DNA, 321 bp, synthetic construct
  misc_feature 1..321: note = Nucleotide sequence of cDNA encoding the variable region of the light chain of antibody 7, 8, and 9
  source 1..321: mol_type = other DNA
gacatccagatgacccagtccccctcctccctctccgcctccgtcggcgaccgcgtcaccatcacctgctccgcctcccagggcatcaacaactacctcaactggtaccagcagaagcccggcaaggcccccaagctcctcatctactacacctccaccctccagtccggcgtcccctcccgcttctccggctccggctccggcaccgacttcaccctcaccatctcctccctccagcccgaggacttcgccacctactactgccagcagtactccaagctcccccgcaccttcggcggcggcaccaaggtcgagatcaag

SEQ ID NO: 24 - protein, 107 aa, synthetic construct
  REGION 1..107: note = Amino acid sequence of the variable region of the light chain of antibody 7, 8 and 9
DIQMTQSPSSLSASVGDRVTITCSASQGINNYLNWYQQKPGKAPKLLIYYTSTLQSGVPSRFSGSGSGTDFTLTISSLQPEDFATYYCQQYSKLPRTFGGGTKVEIK

SEQ ID NO: 25 - DNA, 1353 bp, synthetic construct
  misc_feature 1..1353: note = Nucleotide sequence of the heavy chain of antibody 1
  source 1..1353: mol_type = other DNA
caggttcagctgcagcagtctggcagcgagcttatgatgcctggcgcctccgtgaagatcagctgtaaagccaccggctacaccttcagcaactactggatcgagtgggtcaagcagaggcctggccatggactggaatggatcggagagatcctgcctggcaccggcagaaccatctacaacgagaagttcaagggcaaagccaccttcaccgccgacatcagcagcaacacagtgcagatgcagctgagcagcctgaccagcgaagatagcgccgtgtactactgcgccagacgggactactacggcaacttctactacgccatggattactggggccagggcaccctggttacagtgtctagcgccagcacaaagggcccctccgtgtttccactggctcctagcagcaagagcacaagcggaggaacagccgctctgggctgtctggtcaaggactactttcccgagcctgtgaccgtgtcctggaattctggcgctctgacaagcggcgtgcacacctttccagctgtgctgcaaagcagcggcctgtactctctgagcagcgtggtcacagtgccaagctctagcctgggcacccagacctacatctgcaatgtgaaccacaagcctagcaacaccaaggtggacaagaaggtggaacccaagagctgcgacaagacccacacctgtcctccatgtcctgctccagaactgctcggcggaccctctgtgttcctgtttcctccaaagcctaaggacaccctgatgatcagcagaacccctgaagtgacctgcgtggtggtggatgtgtcccacgaggatcccgaagtgaagttcaattggtacgtggacggcgtggaagtgcacaacgccaagaccaagcctagagaggaacagtacaacagcacctacagagtggtgtccgtgctgaccgtgctgcaccaggattggctgaacggcaaagagtacaagtgcaaggtgtccaacaaggccctgcctgctcctatcgagaaaaccatcagcaaggccaagggccagcctagggaaccccaggtttacacactgcctccaagccgggaagagatgaccaagaaccaggtgtccctgacctgcctcgtgaagggcttctacccttccgatatcgccgtggaatgggagagcaatggccagcctgagaacaactacaagacaacccctcctgtgctggacagcgacggctcattcttcctgtacagcaagctgacagtggacaagtccagatggcagcagggcaacgtgttctcctgcagcgtgatgcacgaggccctgcacaaccactacacccagaagtccctgagcctgtctcctggc

SEQ ID NO: 26 - protein, 451 aa, synthetic construct
  REGION 1..451: note = Amino acid sequence of heavy chain of antibody 1
QVQLQQSGSELMMPGASVKISCKATGYTFSNYWIEWVKQRPGHGLEWIGEILPGTGRTIYNEKFKGKATFTADISSNTVQMQLSSLTSEDSAVYYCARRDYYGNFYYAMDYWGQGTLVTVSSASTKGPSVFPLAPSSKSTSGGTAALGCLVKDYFPEPVTVSWNSGALTSGVHTFPAVLQSSGLYSLSSVVTVPSSSLGTQTYICNVNHKPSNTKVDKKVEPKSCDKTHTCPPCPAPELLGGPSVFLFPPKPKDTLMISRTPEVTCVVVDVSHEDPEVKFNWYVDGVEVHNAKTKPREEQYNSTYRVVSVLTVLHQDWLNGKEYKCKVSNKALPAPIEKTISKAKGQPREPQVYTLPPSREEMTKNQVSLTCLVKGFYPSDIAVEWESNGQPENNYKTTPPVLDSDGSFFLYSKLTVDKSRWQQGNVFSCSVMHEALHNHYTQKSLSLSPG

SEQ ID NO: 27 - DNA, 642 bp, synthetic construct
  misc_feature 1..642: note = Nucleotide sequence of the light chain of antibody 1 and antibody 2
  source 1..642: mol_type = other DNA
gacatccagatgacccagagcaccagcagcctgtctgcctctctgggcgatagagtgaccatcagctgtagcgccagccagggcatcaacaactacctgaactggtatcagcagaaacccgacggcaccgtggaactgctgatctactacaccagcacactgcagagcggcgtgcccagcagattttctggctctggcagcggcaccgactacagcctgacaatcagcaacctggaacctgaggacatcggcacctactactgccagcagtacagcaagctgcccagaacctttggcggaggcaccaagctggaaatcaagcggacagtggccgctcctagcgtgttcatctttccacctagcgacgagcagctgaagtctggcacagcctctgtcgtgtgcctgctgaacaacttctaccccagagaagccaaggtgcagtggaaggtggacaacgccctgcagtccggcaatagccaagagagcgtgaccgagcaggactccaaggacagcacctatagcctgagcagcaccctgacactgagcaaggccgactacgagaagcacaaagtgtacgcctgcgaagtgacccaccagggcctttctagccctgtgaccaagagcttcaaccggggcgagtgt

SEQ ID NO: 28 - protein, 214 aa, synthetic construct
  REGION 1..214: note = Amino acid sequence of the light chain of antibody 1 and antibody 2
DIQMTQSTSSLSASLGDRVTISCSASQGINNYLNWYQQKPDGTVELLIYYTSTLQSGVPSRFSGSGSGTDYSLTISNLEPEDIGTYYCQQYSKLPRTFGGGTKLEIKRTVAAPSVFIFPPSDEQLKSGTASVVCLLNNFYPREAKVQWKVDNALQSGNSQESVTEQDSKDSTYSLSSTLTLSKADYEKHKVYACEVTHQGLSSPVTKSFNRGEC

SEQ ID NO: 29 - DNA, 1347 bp, synthetic construct
  misc_feature 1..1347: note = Nucleotide sequence of the heavy chain of antibody 2
  source 1..1347: mol_type = other DNA
caggttcagctgcagcagtctggcagcgagcttatgatgcctggcgcctccgtgaagatcagctgtaaagccaccggctacaccttcagcaactactggatcgagtgggtcaagcagaggcctggccatggactggaatggatcggagagatcctgcctggcaccggcagaaccatctacaacgagaagttcaagggcaaagccaccttcaccgccgacatcagcagcaacacagtgcagatgcagctgagcagcctgaccagcgaagatagcgccgtgtactactgcgccagacgggactactacggcaacttctactacgccatggattactggggccagggcaccagcgtgacagtgtctagcgcctctacaaagggacccagcgtgttccctctggctccttgtagcagaagcaccagcgagtctacagccgctctgggctgtctggtcaaggactactttcccgagcctgtgaccgtgtcctggaattctggcgctctgacaagcggcgtgcacacctttccagctgtgctgcaaagcagcggcctgtactctctgagcagcgtggtcacagtgcctagctctagcctgggcaccaagacctacacctgtaatgtggaccacaagcctagcaacaccaaggtggacaagcgcgtggaatctaagtacggccctccttgtcctagctgccccgctcctgaatttctcggcggaccttccgtgttcctgtttcctccaaagcctaaggacaccctgatgatcagcagaacccctgaagtgacctgcgtggtggtggacgtgtcccaagaggatcctgaggtgcagttcaattggtacgtggacggcgtggaagtgcacaacgccaagaccaagcctagagaggaacagttcaacagcacctacagagtggtgtccgtgctgaccgtgctgcaccaggattggctgaacggcaaagagtacaagtgcaaggtgtccaacaagggcctgcctagcagcatcgagaaaaccatcagcaaggccaagggccagccaagagaaccccaggtgtacacactgcctccaagccaagaggaaatgaccaagaaccaggtgtccctgacctgcctcgtgaagggcttctacccttccgatatcgccgtggaatgggagagcaatggccagcctgagaacaactacaagacaacccctcctgtgctggacagcgacggctcattcttcctgtacagcagactgaccgtggacaagagcagatggcaagagggcaacgtgttctcctgcagcgtgatgcacgaggccctgcacaaccactacacccagaagtctctgagcctgtctctgggcaag

SEQ ID NO: 30 - protein, 449 aa, synthetic construct
  REGION 1..449: note = Amino acid sequence of heavy chain of antibody 2
QVQLQQSGSELMMPGASVKISCKATGYTFSNYWIEWVKQRPGHGLEWIGEILPGTGRTIYNEKFKGKATFTADISSNTVQMQLSSLTSEDSAVYYCARRDYYGNFYYAMDYWGQGTSVTVSSASTKGPSVFPLAPCSRSTSESTAALGCLVKDYFPEPVTVSWNSGALTSGVHTFPAVLQSSGLYSLSSVVTVPSSSLGTKTYTCNVDHKPSNTKVDKRVESKYGPPCPSCPAPEFLGGPSVFLFPPKPKDTLMISRTPEVTCVVVDVSQEDPEVQFNWYVDGVEVHNAKTKPREEQFNSTYRVVSVLTVLHQDWLNGKEYKCKVSNKGLPSSIEKTISKAKGQPREPQVYTLPPSQEEMTKNQVSLTCLVKGFYPSDIAVEWESNGQPENNYKTTPPVLDSDGSFFLYSRLTVDKSRWQEGNVFSCSVMHEALHNHYTQKSLSLSLGK

SEQ ID NO: 31 - DNA, 1353 bp, synthetic construct
  misc_feature 1..1353: note = Nucleotide sequence of the heavy chain of antibody 3
  source 1..1353: mol_type = other DNA
caggtccagctcgtccagtccggcgccgaggtcaagaagcccggctcctccgtcaaggtctcctgcaaggcctccggctacaccttctccaactactggatcgagtgggtccgccaggcccccggccagggcctcgagtggatcggcgagatcctccccggcaccggccgcaccatctacaacgagaagttcaagggccgcgccaccttcaccgccgacatctccacctccaccgcctacatggagctctcctccctccgctccgaggacaccgccgtctactactgcgcccgccgcgactactacggcaacttctactacgccatggactactggggccagggcaccctcgtcaccgtctcctccgcctccaccaagggcccctccgtcttccccctcgccccctcctccaagtccacctccggcggcaccgccgccctcggctgcctcgtcaaggactacttccccgagcccgtcaccgtctcctggaactccggcgccctcacctccggcgtccacaccttccccgccgtcctccagtcctccggcctctactccctctcctccgtcgtcaccgtcccctcctcctccctcggcacccagacctacatctgcaacgtcaaccacaagccctccaacaccaaggtcgacaagaaggtcgagcccaagtcctgcgacaagacccacacctgccccccctgccccgcccccgaggccgccggcggcccctccgtcttcctcttcccccccaagcccaaggacaccctcatgatctcccgcacccccgaggtcacctgcgtcgtcgtcgacgtctcccacgaggaccccgaggtcaagttcaactggtacgtcgacggcgtcgaggtccacaacgccaagaccaagccccgcgaggagcagtacaactccacctaccgcgtcgtctccgtcctcaccgtcctccaccaggactggctcaacggcaaggagtacaagtgcaaggtctccaacaaggccctccccgcccccatcgagaagaccatctccaaggccaagggccagccccgcgagccccaggtctacaccctccccccctcccgcgaggagatgaccaagaaccaggtctccctcacctgcctcgtcaagggcttctacccctccgacatcgccgtcgagtgggagtccaacggccagcccgagaacaactacaagaccaccccccccgtcctcgactccgacggctccttcttcctctactccaagctcaccgtcgacaagtcccgctggcagcagggcaacgtcttctcctgctccgtcatgcacgaggccctccacaaccactacacccagaagtccctctccctctcccccggc

SEQ ID NO: 32 - protein, 451 aa, synthetic construct
  REGION 1..451: note = Amino acid sequence of heavy chain of antibody 3
QVQLVQSGAEVKKPGSSVKVSCKASGYTFSNYWIEWVRQAPGQGLEWIGEILPGTGRTIYNEKFKGRATFTADISTSTAYMELSSLRSEDTAVYYCARRDYYGNFYYAMDYWGQGTLVTVSSASTKGPSVFPLAPSSKSTSGGTAALGCLVKDYFPEPVTVSWNSGALTSGVHTFPAVLQSSGLYSLSSVVTVPSSSLGTQTYICNVNHKPSNTKVDKKVEPKSCDKTHTCPPCPAPEAAGGPSVFLFPPKPKDTLMISRTPEVTCVVVDVSHEDPEVKFNWYVDGVEVHNAKTKPREEQYNSTYRVVSVLTVLHQDWLNGKEYKCKVSNKALPAPIEKTISKAKGQPREPQVYTLPPSREEMTKNQVSLTCLVKGFYPSDIAVEWESNGQPENNYKTTPPVLDSDGSFFLYSKLTVDKSRWQQGNVFSCSVMHEALHNHYTQKSLSLSPG

SEQ ID NO: 33 - DNA, 642 bp, synthetic construct
  misc_feature 1..642: note = Nucleotide sequence of the light chain of antibody 3, 4, 5, 6, 10, 11, and 12
  source 1..642: mol_type = other DNA
gacatccagatgacccagtccccctcctccctctccgcctccgtcggcgaccgcgtcaccatcacctgctccgcctcccagggcatcaacaactacctcaactggtaccagcagaagcccggcaaggcccccaagctcctcatctactacacctccaccctccagtccggcgtcccctcccgcttctccggctccggctccggcaccgactacaccctcaccatctcctccctccagcccgaggacttcgccacctactactgccagcagtactccaagctcccccgcaccttcggcggcggcaccaaggtcgagatcaagcgcaccgtcgccgccccctccgtcttcatcttccccccctccgacgagcagctcaagtccggcaccgcctccgtcgtctgcctcctcaacaacttctacccccgcgaggccaaggtccagtggaaggtcgacaacgccctccagtccggcaactcccaggagtccgtcaccgagcaggactccaaggactccacctactccctctcctccaccctcaccctctccaaggccgactacgagaagcacaaggtctacgcctgcgaggtcacccaccagggcctctcctcccccgtcaccaagtccttcaaccgcggcgagtgc

SEQ ID NO: 34 - protein, 214 aa, synthetic construct
  REGION 1..214: note = Amino acid sequence of the light chain of antibody 3, 4, 5, 6, 10, 11, and 12
DIQMTQSPSSLSASVGDRVTITCSASQGINNYLNWYQQKPGKAPKLLIYYTSTLQSGVPSRFSGSGSGTDYTLTISSLQPEDFATYYCQQYSKLPRTFGGGTKVEIKRTVAAPSVFIFPPSDEQLKSGTASVVCLLNNFYPREAKVQWKVDNALQSGNSQESVTEQDSKDSTYSLSSTLTLSKADYEKHKVYACEVTHQGLSSPVTKSFNRGEC

SEQ ID NO: 35 - DNA, 1353 bp, synthetic construct
  misc_feature 1..1353: note = Nucleotide sequence of the heavy chain of antibody 4 and antibody 7
  source 1..1353: mol_type = other DNA
caggtccagctcgtccagtccggcgccgaggtcaagaagcccggctcctccgtcaaggtctcctgcaaggcctccggctacaccttctccaactactggatcgagtgggtccgccaggcccccggccagggcctcgagtggatcggcgagatcctccccggcaccggccgcaccatctacaacgagaagttcaagggccgcgtcaccttcaccgccgacatctccacctccaccgcctacatggagctctcctccctccgctccgaggacaccgccgtctactactgcgcccgccgcgactactacggcaacttctactacgccatggactactggggccagggcaccctcgtcaccgtctcctccgcctccaccaagggcccctccgtcttccccctcgccccctcctccaagtccacctccggcggcaccgccgccctcggctgcctcgtcaaggactacttccccgagcccgtcaccgtctcctggaactccggcgccctcacctccggcgtccacaccttccccgccgtcctccagtcctccggcctctactccctctcctccgtcgtcaccgtcccctcctcctccctcggcacccagacctacatctgcaacgtcaaccacaagccctccaacaccaaggtcgacaagaaggtcgagcccaagtcctgcgacaagacccacacctgccccccctgccccgcccccgaggccgccggcggcccctccgtcttcctcttcccccccaagcccaaggacaccctcatgatctcccgcacccccgaggtcacctgcgtcgtcgtcgacgtctcccacgaggaccccgaggtcaagttcaactggtacgtcgacggcgtcgaggtccacaacgccaagaccaagccccgcgaggagcagtacaactccacctaccgcgtcgtctccgtcctcaccgtcctccaccaggactggctcaacggcaaggagtacaagtgcaaggtctccaacaaggccctccccgcccccatcgagaagaccatctccaaggccaagggccagccccgcgagccccaggtctacaccctccccccctcccgcgaggagatgaccaagaaccaggtctccctcacctgcctcgtcaagggcttctacccctccgacatcgccgtcgagtgggagtccaacggccagcccgagaacaactacaagaccaccccccccgtcctcgactccgacggctccttcttcctctactccaagctcaccgtcgacaagtcccgctggcagcagggcaacgtcttctcctgctccgtcatgcacgaggccctccacaaccactacacccagaagtccctctccctctcccccggc

SEQ ID NO: 36 - protein, 451 aa, synthetic construct
  REGION 1..451: note = Amino acid sequence of heavy chain of antibody 4 and antibody 7
QVQLVQSGAEVKKPGSSVKVSCKASGYTFSNYWIEWVRQAPGQGLEWIGEILPGTGRTIYNEKFKGRVTFTADISTSTAYMELSSLRSEDTAVYYCARRDYYGNFYYAMDYWGQGTLVTVSSASTKGPSVFPLAPSSKSTSGGTAALGCLVKDYFPEPVTVSWNSGALTSGVHTFPAVLQSSGLYSLSSVVTVPSSSLGTQTYICNVNHKPSNTKVDKKVEPKSCDKTHTCPPCPAPEAAGGPSVFLFPPKPKDTLMISRTPEVTCVVVDVSHEDPEVKFNWYVDGVEVHNAKTKPREEQYNSTYRVVSVLTVLHQDWLNGKEYKCKVSNKALPAPIEKTISKAKGQPREPQVYTLPPSREEMTKNQVSLTCLVKGFYPSDIAVEWESNGQPENNYKTTPPVLDSDGSFFLYSKLTVDKSRWQQGNVFSCSVMHEALHNHYTQKSLSLSPG

SEQ ID NO: 37 - DNA, 1353 bp, synthetic construct
  misc_feature 1..1353: note = Nucleotide sequence of the heavy chain of antibody 5 and antibody 8
  source 1..1353: mol_type = other DNA
caggtccagctcgtccagtccggcgccgaggtcaagaagcccggctcctccgtcaaggtctcctgcaaggcctccggctacaccttctccaactactggatcgagtgggtccgccaggcccccggccagggcctcgagtggatcggcgagatcctccccggcaccggccgcaccatctacaacgagaagttcaagggccgcgccaccttcaccgccgacgagtccacctccaccgcctacatggagctctcctccctccgctccgaggacaccgccgtctactactgcgcccgccgcgactactacggcaacttctactacgccatggactactggggccagggcaccctcgtcaccgtctcctccgcctccaccaagggcccctccgtcttccccctcgccccctcctccaagtccacctccggcggcaccgccgccctcggctgcctcgtcaaggactacttccccgagcccgtcaccgtctcctggaactccggcgccctcacctccggcgtccacaccttccccgccgtcctccagtcctccggcctctactccctctcctccgtcgtcaccgtcccctcctcctccctcggcacccagacctacatctgcaacgtcaaccacaagccctccaacaccaaggtcgacaagaaggtcgagcccaagtcctgcgacaagacccacacctgccccccctgccccgcccccgaggccgccggcggcccctccgtcttcctcttcccccccaagcccaaggacaccctcatgatctcccgcacccccgaggtcacctgcgtcgtcgtcgacgtctcccacgaggaccccgaggtcaagttcaactggtacgtcgacggcgtcgaggtccacaacgccaagaccaagccccgcgaggagcagtacaactccacctaccgcgtcgtctccgtcctcaccgtcctccaccaggactggctcaacggcaaggagtacaagtgcaaggtctccaacaaggccctccccgcccccatcgagaagaccatctccaaggccaagggccagccccgcgagccccaggtctacaccctccccccctcccgcgaggagatgaccaagaaccaggtctccctcacctgcctcgtcaagggcttctacccctccgacatcgccgtcgagtgggagtccaacggccagcccgagaacaactacaagaccaccccccccgtcctcgactccgacggctccttcttcctctactccaagctcaccgtcgacaagtcccgctggcagcagggcaacgtcttctcctgctccgtcatgcacgaggccctccacaaccactacacccagaagtccctctccctctcccccggc

SEQ ID NO: 38 - protein, 451 aa, synthetic construct
  REGION 1..451: note = Amino acid sequence of heavy chain of antibody 5 and antibody 8
QVQLVQSGAEVKKPGSSVKVSCKASGYTFSNYWIEWVRQAPGQGLEWIGEILPGTGRTIYNEKFKGRATFTADESTSTAYMELSSLRSEDTAVYYCARRDYYGNFYYAMDYWGQGTLVTVSSASTKGPSVFPLAPSSKSTSGGTAALGCLVKDYFPEPVTVSWNSGALTSGVHTFPAVLQSSGLYSLSSVVTVPSSSLGTQTYICNVNHKPSNTKVDKKVEPKSCDKTHTCPPCPAPEAAGGPSVFLFPPKPKDTLMISRTPEVTCVVVDVSHEDPEVKFNWYVDGVEVHNAKTKPREEQYNSTYRVVSVLTVLHQDWLNGKEYKCKVSNKALPAPIEKTISKAKGQPREPQVYTLPPSREEMTKNQVSLTCLVKGFYPSDIAVEWESNGQPENNYKTTPPVLDSDGSFFLYSKLTVDKSRWQQGNVFSCSVMHEALHNHYTQKSLSLSPG

SEQ ID NO: 39 - DNA, 1353 bp, synthetic construct
  misc_feature 1..1353: note = Nucleotide sequence of the heavy chain of antibody 6 and antibody 9
  source 1..1353: mol_type = other DNA
caggtccagctcgtccagtccggcgccgaggtcaagaagcccggctcctccgtcaaggtctcctgcaaggcctccggctacaccttctccaactactggatcgagtgggtccgccaggcccccggccagggcctcgagtggatcggcgagatcctccccggcaccggccgcaccatctacaacgagaagttcaagggccgcgtcaccttcaccgccgacgagtccacctccaccgcctacatggagctctcctccctccgctccgaggacaccgccgtctactactgcgcccgccgcgactactacggcaacttctactacgccatggactactggggccagggcaccctcgtcaccgtctcctccgcctccaccaagggcccctccgtcttccccctcgccccctcctccaagtccacctccggcggcaccgccgccctcggctgcctcgtcaaggactacttccccgagcccgtcaccgtctcctggaactccggcgccctcacctccggcgtccacaccttccccgccgtcctccagtcctccggcctctactccctctcctccgtcgtcaccgtcccctcctcctccctcggcacccagacctacatctgcaacgtcaaccacaagccctccaacaccaaggtcgacaagaaggtcgagcccaagtcctgcgacaagacccacacctgccccccctgccccgcccccgaggccgccggcggcccctccgtcttcctcttcccccccaagcccaaggacaccctcatgatctcccgcacccccgaggtcacctgcgtcgtcgtcgacgtctcccacgaggaccccgaggtcaagttcaactggtacgtcgacggcgtcgaggtccacaacgccaagaccaagccccgcgaggagcagtacaactccacctaccgcgtcgtctccgtcctcaccgtcctccaccaggactggctcaacggcaaggagtacaagtgcaaggtctccaacaaggccctccccgcccccatcgagaagaccatctccaaggccaagggccagccccgcgagccccaggtctacaccctccccccctcccgcgaggagatgaccaagaaccaggtctccctcacctgcctcgtcaagggcttctacccctccgacatcgccgtcgagtgggagtccaacggccagcccgagaacaactacaagaccaccccccccgtcctcgactccgacggctccttcttcctctactccaagctcaccgtcgacaagtcccgctggcagcagggcaacgtcttctcctgctccgtcatgcacgaggccctccacaaccactacacccagaagtccctctccctctcccccggc

SEQ ID NO: 40 - protein, 451 aa, synthetic construct
  REGION 1..451: note = Amino acid sequence of the heavy chain of antibody 6 and antibody 9
QVQLVQSGAEVKKPGSSVKVSCKASGYTFSNYWIEWVRQAPGQGLEWIGEILPGTGRTIYNEKFKGRVTFTADESTSTAYMELSSLRSEDTAVYYCARRDYYGNFYYAMDYWGQGTLVTVSSASTKGPSVFPLAPSSKSTSGGTAALGCLVKDYFPEPVTVSWNSGALTSGVHTFPAVLQSSGLYSLSSVVTVPSSSLGTQTYICNVNHKPSNTKVDKKVEPKSCDKTHTCPPCPAPEAAGGPSVFLFPPKPKDTLMISRTPEVTCVVVDVSHEDPEVKFNWYVDGVEVHNAKTKPREEQYNSTYRVVSVLTVLHQDWLNGKEYKCKVSNKALPAPIEKTISKAKGQPREPQVYTLPPSREEMTKNQVSLTCLVKGFYPSDIAVEWESNGQPENNYKTTPPVLDSDGSFFLYSKLTVDKSRWQQGNVFSCSVMHEALHNHYTQKSLSLSPG

SEQ ID NO: 41 - DNA, 642 bp, synthetic construct
  misc_feature 1..642: note = Nucleotide sequence of the light chain of antibody 7, 8 and 9
  source 1..642: mol_type = other DNA
gacatccagatgacccagtccccctcctccctctccgcctccgtcggcgaccgcgtcaccatcacctgctccgcctcccagggcatcaacaactacctcaactggtaccagcagaagcccggcaaggcccccaagctcctcatctactacacctccaccctccagtccggcgtcccctcccgcttctccggctccggctccggcaccgacttcaccctcaccatctcctccctccagcccgaggacttcgccacctactactgccagcagtactccaagctcccccgcaccttcggcggcggcaccaaggtcgagatcaagcgcaccgtcgccgccccctccgtcttcatcttccccccctccgacgagcagctcaagtccggcaccgcctccgtcgtctgcctcctcaacaacttctacccccgcgaggccaaggtccagtggaaggtcgacaacgccctccagtccggcaactcccaggagtccgtcaccgagcaggactccaaggactccacctactccctctcctccaccctcaccctctccaaggccgactacgagaagcacaaggtctacgcctgcgaggtcacccaccagggcctctcctcccccgtcaccaagtccttcaaccgcggcgagtgc

SEQ ID NO: 42 - protein, 214 aa, synthetic construct
  REGION 1..214: note = Amino acid sequence of the light chain of antibody 7, 8 and 9
DIQMTQSPSSLSASVGDRVTITCSASQGINNYLNWYQQKPGKAPKLLIYYTSTLQSGVPSRFSGSGSGTDFTLTISSLQPEDFATYYCQQYSKLPRTFGGGTKVEIKRTVAAPSVFIFPPSDEQLKSGTASVVCLLNNFYPREAKVQWKVDNALQSGNSQESVTEQDSKDSTYSLSSTLTLSKADYEKHKVYACEVTHQGLSSPVTKSFNRGEC

SEQ ID NO: 43 - DNA, 1353 bp, synthetic construct
  misc_feature 1..1353: note = Nucleotide sequence of the heavy chain of antibody 10
  source 1..1353: mol_type = other DNA
caggtccagctcgtccagtccggcgccgaggtcaagaagcccggctcctccgtcaaggtctcctgcaaggcctccggctacaccttctccaactactggatcgagtgggtccgccaggcccccggccagggcctcgagtggatcggcgagatcctccccggcaccggccgcaccatctacaacgagaagttcaagggccgcgccaccttcaccgccgacatctccacctccaccgcctacatggagctctcctccctccgctccgaggacaccgccgtctactactgcgcccgccgcgactactacggcaacttctactacgccatggactactggggccagggcaccctcgtcaccgtctcctccgcctccaccaagggcccctccgtcttccccctcgccccctcctccaagtccacctccggcggcaccgccgccctcggctgcctcgtcaaggactacttccccgagcccgtcaccgtctcctggaactccggcgccctcacctccggcgtccacaccttccccgccgtcctccagtcctccggcctctactccctctcctccgtcgtcaccgtcccctcctcctccctcggcacccagacctacatctgcaacgtcaaccacaagccctccaacaccaaggtcgacaagaaggtcgagcccaagtcctgcgacaagacccacacctgccccccctgccccgcccccgagctcctcggcggcccctccgtcttcctcttcccccccaagcccaaggacaccctcatgatctcccgcacccccgaggtcacctgcgtcgtcgtcgacgtctcccacgaggaccccgaggtcaagttcaactggtacgtcgacggcgtcgaggtccacaacgccaagaccaagccccgcgaggagcagtacaactccacctaccgcgtcgtctccgtcctcaccgtcctccaccaggactggctcaacggcaaggagtacaagtgcaaggtctccaacaaggccctccccgcccccatcgagaagaccatctccaaggccaagggccagccccgcgagccccaggtctacaccctccccccctcccgcgaggagatgaccaagaaccaggtctccctcacctgcctcgtcaagggcttctacccctccgacatcgccgtcgagtgggagtccaacggccagcccgagaacaactacaagaccaccccccccgtcctcgactccgacggctccttcttcctctactccaagctcaccgtcgacaagtcccgctggcagcagggcaacgtcttctcctgctccgtcatgcacgaggccctccacaaccactacacccagaagtccctctccctctcccccggc

SEQ ID NO: 44 - protein, 451 aa, synthetic construct
  REGION 1..451: note = Amino acid sequence of the heavy chain of antibody 10
QVQLVQSGAEVKKPGSSVKVSCKASGYTFSNYWIEWVRQAPGQGLEWIGEILPGTGRTIYNEKFKGRATFTADISTSTAYMELSSLRSEDTAVYYCARRDYYGNFYYAMDYWGQGTLVTVSSASTKGPSVFPLAPSSKSTSGGTAALGCLVKDYFPEPVTVSWNSGALTSGVHTFPAVLQSSGLYSLSSVVTVPSSSLGTQTYICNVNHKPSNTKVDKKVEPKSCDKTHTCPPCPAPELLGGPSVFLFPPKPKDTLMISRTPEVTCVVVDVSHEDPEVKFNWYVDGVEVHNAKTKPREEQYNSTYRVVSVLTVLHQDWLNGKEYKCKVSNKALPAPIEKTISKAKGQPREPQVYTLPPSREEMTKNQVSLTCLVKGFYPSDIAVEWESNGQPENNYKTTPPVLDSDGSFFLYSKLTVDKSRWQQGNVFSCSVMHEALHNHYTQKSLSLSPG

SEQ ID NO: 45 - DNA, 1353 bp, synthetic construct
  misc_feature 1..1353: note = Nucleotide sequence of the heavy chain of antibody 11
  source 1..1353: mol_type = other DNA
caggtccagctcgtccagtccggcgccgaggtcaagaagcccggctcctccgtcaaggtctcctgcaaggcctccggctacaccttctccaactactggatcgagtgggtccgccaggcccccggccagggcctcgagtggatcggcgagatcctccccggcaccggccgcaccatctacaacgagaagttcaagggccgcgtcaccttcaccgccgacatctccacctccaccgcctacatggagctctcctccctccgctccgaggacaccgccgtctactactgcgcccgccgcgactactacggcaacttctactacgccatggactactggggccagggcaccctcgtcaccgtctcctccgcctccaccaagggcccctccgtcttccccctcgccccctcctccaagtccacctccggcggcaccgccgccctcggctgcctcgtcaaggactacttccccgagcccgtcaccgtctcctggaactccggcgccctcacctccggcgtccacaccttccccgccgtcctccagtcctccggcctctactccctctcctccgtcgtcaccgtcccctcctcctccctcggcacccagacctacatctgcaacgtcaaccacaagccctccaacaccaaggtcgacaagaaggtcgagcccaagtcctgcgacaagacccacacctgccccccctgccccgcccccgagctcctcggcggcccctccgtcttcctcttcccccccaagcccaaggacaccctcatgatctcccgcacccccgaggtcacctgcgtcgtcgtcgacgtctcccacgaggaccccgaggtcaagttcaactggtacgtcgacggcgtcgaggtccacaacgccaagaccaagccccgcgaggagcagtacaactccacctaccgcgtcgtctccgtcctcaccgtcctccaccaggactggctcaacggcaaggagtacaagtgcaaggtctccaacaaggccctccccgcccccatcgagaagaccatctccaaggccaagggccagccccgcgagccccaggtctacaccctccccccctcccgcgaggagatgaccaagaaccaggtctccctcacctgcctcgtcaagggcttctacccctccgacatcgccgtcgagtgggagtccaacggccagcccgagaacaactacaagaccaccccccccgtcctcgactccgacggctccttcttcctctactccaagctcaccgtcgacaagtcccgctggcagcagggcaacgtcttctcctgctccgtcatgcacgaggccctccacaaccactacacccagaagtccctctccctctcccccggc

SEQ ID NO: 46 - protein, 451 aa, synthetic construct
  REGION 1..451: note = Amino acid sequence of the heavy chain of antibody 11
QVQLVQSGAEVKKPGSSVKVSCKASGYTFSNYWIEWVRQAPGQGLEWIGEILPGTGRTIYNEKFKGRVTFTADISTSTAYMELSSLRSEDTAVYYCARRDYYGNFYYAMDYWGQGTLVTVSSASTKGPSVFPLAPSSKSTSGGTAALGCLVKDYFPEPVTVSWNSGALTSGVHTFPAVLQSSGLYSLSSVVTVPSSSLGTQTYICNVNHKPSNTKVDKKVEPKSCDKTHTCPPCPAPELLGGPSVFLFPPKPKDTLMISRTPEVTCVVVDVSHEDPEVKFNWYVDGVEVHNAKTKPREEQYNSTYRVVSVLTVLHQDWLNGKEYKCKVSNKALPAPIEKTISKAKGQPREPQVYTLPPSREEMTKNQVSLTCLVKGFYPSDIAVEWESNGQPENNYKTTPPVLDSDGSFFLYSKLTVDKSRWQQGNVFSCSVMHEALHNHYTQKSLSLSPG

SEQ ID NO: 47 - DNA, 1353 bp, synthetic construct
  misc_feature 1..1353: note = Nucleotide sequence of the heavy chain of antibody 12
  source 1..1353: mol_type = other DNA
caggtccagctcgtccagtccggcgccgaggtcaagaagcccggctcctccgtcaaggtctcctgcaaggcctccggctacaccttctccaactactggatcgagtgggtccgccaggcccccggccagggcctcgagtggatcggcgagatcctccccggcaccggccgcaccatctacaacgagaagttcaagggccgcgtcaccttcaccgccgacgagtccacctccaccgcctacatggagctctcctccctccgctccgaggacaccgccgtctactactgcgcccgccgcgactactacggcaacttctactacgccatggactactggggccagggcaccctcgtcaccgtctcctccgcctccaccaagggcccctccgtcttccccctcgccccctcctccaagtccacctccggcggcaccgccgccctcggctgcctcgtcaaggactacttccccgagcccgtcaccgtctcctggaactccggcgccctcacctccggcgtccacaccttccccgccgtcctccagtcctccggcctctactccctctcctccgtcgtcaccgtcccctcctcctccctcggcacccagacctacatctgcaacgtcaaccacaagccctccaacaccaaggtcgacaagaaggtcgagcccaagtcctgcgacaagacccacacctgccccccctgccccgcccccgagctcctcggcggcccctccgtcttcctcttcccccccaagcccaaggacaccctcatgatctcccgcacccccgaggtcacctgcgtcgtcgtcgacgtctcccacgaggaccccgaggtcaagttcaactggtacgtcgacggcgtcgaggtccacaacgccaagaccaagccccgcgaggagcagtacaactccacctaccgcgtcgtctccgtcctcaccgtcctccaccaggactggctcaacggcaaggagtacaagtgcaaggtctccaacaaggccctccccgcccccatcgagaagaccatctccaaggccaagggccagccccgcgagccccaggtctacaccctccccccctcccgcgaggagatgaccaagaaccaggtctccctcacctgcctcgtcaagggcttctacccctccgacatcgccgtcgagtgggagtccaacggccagcccgagaacaactacaagaccaccccccccgtcctcgactccgacggctccttcttcctctactccaagctcaccgtcgacaagtcccgctggcagcagggcaacgtcttctcctgctccgtcatgcacgaggccctccacaaccactacacccagaagtccctctccctctcccccggc

SEQ ID NO: 48 - protein, 451 aa, synthetic construct
  REGION 1..451: note = Amino acid sequence of the heavy chain of antibody 12
QVQLVQSGAEVKKPGSSVKVSCKASGYTFSNYWIEWVRQAPGQGLEWIGEILPGTGRTIYNEKFKGRVTFTADESTSTAYMELSSLRSEDTAVYYCARRDYYGNFYYAMDYWGQGTLVTVSSASTKGPSVFPLAPSSKSTSGGTAALGCLVKDYFPEPVTVSWNSGALTSGVHTFPAVLQSSGLYSLSSVVTVPSSSLGTQTYICNVNHKPSNTKVDKKVEPKSCDKTHTCPPCPAPELLGGPSVFLFPPKPKDTLMISRTPEVTCVVVDVSHEDPEVKFNWYVDGVEVHNAKTKPREEQYNSTYRVVSVLTVLHQDWLNGKEYKCKVSNKALPAPIEKTISKAKGQPREPQVYTLPPSREEMTKNQVSLTCLVKGFYPSDIAVEWESNGQPENNYKTTPPVLDSDGSFFLYSKLTVDKSRWQQGNVFSCSVMHEALHNHYTQKSLSLSPG

SEQ ID NO: 49 - protein, 310 aa, synthetic construct
  REGION 1..310: note = Amino acid sequence of human CD138 protein
MRRAALWLWLCALALSLQPALPQIVATNLPPEDQDGSGDDSDNFSGSGAGALQDITLSQQTPSTWKDTQLLTAIPTSPEPTGLEATAASTSTLPAGEGPKEGEAVVLPEVEPGLTAREQEATPRPRETTQLPTTHLASTTTATTAQEPATSHPHRDMQPGHHETSTPAGPSQADLHTPHTEDGGPSATERAAEDGASSQLPAAEGSGEQDFTFETSGENTAVVAVEPDRRNQSPVDQGATGASQGLLDRKEVLGGVIAGGLVGLIFAVCLVGFMLYRMKKKDEGSYSLEEPKQANGGAYQKPTKQEEFYA

SEQ ID NO: 50 - protein, 4 aa, synthetic construct
  REGION 1..4: note = Specific epitope sequence in CD138
LPEV